European Patent Specification EP 4 092 115 B1, published July 3, 2024. Title: Novel dihydrolipoamide acetyltransferase variant and a method for producing L-valine using the same. Applicant: CJ CheilJedang Corporation. The sequence listing filed with the application follows.

SEQUENCE LISTING (10 sequences)

SEQ ID NO: 1 - protein, 670 aa, Artificial Sequence
  dihydrolipoamide acetyltransferase variant
MAFSVEMPELGESVTEGTITQWLKSVGDTVEVDEPLLEVSTDKVDTEIPSPVAGVILEIKAEEDDTVDVGGVIAIIDDADETPANEAPADEAPAPAEEEEPVKEEPKKEAAPEAPAATGAATDVEMPELGESVTEGTITQWLKAVGDTVEVDEPLLEVSTDKVDTEIPSPVAGTIVEILADEDDTVDVGAVIARIGDANAAAAPAEEEAAPAEEEEPVKEEPKKEAAPEAPAATGAATDVEMPELGESVTEGTITQWLKAVGDTVEVDEPLLEVSTDKVDTEIPSPVAGTIVEILADEDDTVDVGAVIARIGDANAAAAPGEEKAAPAEEEEPKQEEPKKEEPKKEAATTPAAASATVSASGDNVPYVTPLVRKLAEKHGVDLNTVTGTGIGGRIRKQDVLAAANGEAAPAEAAAPVSAWSTKSVDPEKAKLRGTTQKVNRIREITAMKTVEALQISAQLTQLHEVDMTRVAELRKKNKPAFIEKHGVNLTYLPFFVKAVVEALVSHPNVNASYNAKTKEMTYHSSVNLSIAVDTPAGLLTPVIHDAQDLSIPEIAKAIVDLADRSRNNKLKPNDLSGGTFTITNIGSEGALSDTPILVPPQAGILGTGAIVKRPVVITEDGIDSIAIRQMVFLPLTYDHQVVDGADAGRFLTTIKDRLETANFEGDLQL

SEQ ID NO: 2 - DNA, 2013 bp, Artificial Sequence
  dihydrolipoamide acetyltransferase variant coding gene
atggcgttctccgtagagatgcccgagctgggcgaatcagtaaccgaaggcacgatcacccagtggttgaagtctgttggtgacactgttgaggtagatgagccgttgctcgaggtctcaactgacaaggtcgacaccgagattccctctcctgtcgccggtgtcatcctagagattaaggctgaagaggatgacaccgtcgacgtcggcggtgtcattgcaataatcgacgatgctgatgagactcctgccaacgaagctcctgccgacgaggcaccagctcctgccgaagaggaagaaccagttaaggaagagccaaagaaggaggcagctcctgaagctccagcagcaactggcgccgcaaccgatgtggaaatgccagaactcggcgaatccgtcaccgaaggcaccattacccagtggctcaaggctgtcggcgacaccgtcgaagtagacgaaccacttcttgaggtctccaccgacaaggtcgacaccgaaatcccatctccagtagcaggcaccatcgtggagatccttgcagacgaagacgacaccgtcgacgtcggcgcagtcatcgcccgcatcggtgacgcaaacgcagctgcagcacctgccgaagaggaagcagcacctgccgaagaggaagagccagttaaggaagagccaaagaaggaggcagctcctgaagctccagcagcaactggcgcagcaaccgatgtggaaatgccagaactcggcgaatccgtcaccgaaggcaccattacccagtggctcaaggctgtcggcgacaccgtcgaagtagacgaaccacttcttgaggtctccaccgacaaggtcgacaccgaaatcccatccccagtagcaggcaccatcgtggagatccttgcagacgaagacgacaccgtcgacgtcggcgcagtcatcgcccgcatcggtgacgcaaacgcagctgcagcacctggcgaagagaaagcagcacctgccgaagaggaagagccaaagcaggaagagccaaagaaggaagagccaaagaaggaagcagctactacacctgctgcggcatccgcaactgtgtccgcttctggcgacaacgttccatacgtcaccccactggtgcgcaagcttgctgaaaagcacggcgttgacttgaacaccgtgaccggtaccggtatcggtggccgtatccgcaagcaggatgttttggctgctgcgaacggcgaggctgcacctgctgaggctgctgctcctgtttccgcttggtccactaagtctgttgatcctgagaaggctaagctccgtggtaccactcagaaggtcaaccgcatccgtgagatcaccgcgatgaagaccgtcgaggctctgcagatttctgctcagctcacccagctgcacgaggtcgatatgactcgcgttgctgagctgcgtaagaagaacaagcccgcgttcatcgagaagcacggtgtgaacctcacttacctgccattcttcgtgaaggcagttgtcgaggctttggtttcccatccaaacgtcaacgcgtcttacaacgcgaagaccaaggagatgacctaccactcctccgttaacctctccatcgctgttgataccccagctggtctgttgaccccagtcattcacgatgctcaggatctctccatcccagagatcgcaaaggcaattgttgacctggctgatcgttcacgcaacaacaagctgaagccaaacgatctgtccggtggcaccttcaccatcaccaacattggttctgaaggcgcactgtctgataccccaatcctggttccaccacaggctggcatcttgggcaccggcgcgatcgtgaagcgtccagttgtcatcaccgaggatggaattgattccatcgcgatccgtcagatggtcttcctgccactgacctacgaccaccaggttgtagatggcgcagatgctggtcgcttcctgaccaccatcaaggaccgccttgagaccgctaacttcgaaggcgatctgcagctctaa

SEQ ID NO: 3 - protein, 670 aa, Artificial Sequence
  Wild-type dihydrolipoamide acetyltransferase
MAFSVEMPELGESVTEGTITQWLKSVGDTVEVDEPLLEVSTDKVDTEIPSPVAGVILEIKAEEDDTVDVGGVIAIIGDADETPANEAPADEAPAPAEEEEPVKEEPKKEAAPEAPAATGAATDVEMPELGESVTEGTITQWLKAVGDTVEVDEPLLEVSTDKVDTEIPSPVAGTIVEILADEDDTVDVGAVIARIGDANAAAAPAEEEAAPAEEEEPVKEEPKKEAAPEAPAATGAATDVEMPELGESVTEGTITQWLKAVGDTVEVDEPLLEVSTDKVDTEIPSPVAGTIVEILADEDDTVDVGAVIARIGDANAAAAPGEEKAAPAEEEEPKQEEPKKEEPKKEAATTPAAASATVSASGDNVPYVTPLVRKLAEKHGVDLNTVTGTGIGGRIRKQDVLAAANGEAAPAEAAAPVSAWSTKSVDPEKAKLRGTTQKVNRIREITAMKTVEALQISAQLTQLHEVDMTRVAELRKKNKPAFIEKHGVNLTYLPFFVKAVVEALVSHPNVNASYNAKTKEMTYHSSVNLSIAVDTPAGLLTPVIHDAQDLSIPEIAKAIVDLADRSRNNKLKPNDLSGGTFTITNIGSEGALSDTPILVPPQAGILGTGAIVKRPVVITEDGIDSIAIRQMVFLPLTYDHQVVDGADAGRFLTTIKDRLETANFEGDLQL

SEQ ID NO: 4 - DNA, 2013 bp, Artificial Sequence
  Wild-type dihydrolipoamide acetyltransferase coding gene
atggcgttctccgtagagatgcccgagctgggcgaatcagtaaccgaaggcacgatcacccagtggttgaagtctgttggtgacactgttgaggtagatgagccgttgctcgaggtctcaactgacaaggtcgacaccgagattccctctcctgtcgccggtgtcatcctagagattaaggctgaagaggatgacaccgtcgacgtcggcggtgtcattgcaataatcggcgatgctgatgagactcctgccaacgaagctcctgccgacgaggcaccagctcctgccgaagaggaagaaccagttaaggaagagccaaagaaggaggcagctcctgaagctccagcagcaactggcgccgcaaccgatgtggaaatgccagaactcggcgaatccgtcaccgaaggcaccattacccagtggctcaaggctgtcggcgacaccgtcgaagtagacgaaccacttcttgaggtctccaccgacaaggtcgacaccgaaatcccatctccagtagcaggcaccatcgtggagatccttgcagacgaagacgacaccgtcgacgtcggcgcagtcatcgcccgcatcggtgacgcaaacgcagctgcagcacctgccgaagaggaagcagcacctgccgaagaggaagagccagttaaggaagagccaaagaaggaggcagctcctgaagctccagcagcaactggcgcagcaaccgatgtggaaatgccagaactcggcgaatccgtcaccgaaggcaccattacccagtggctcaaggctgtcggcgacaccgtcgaagtagacgaaccacttcttgaggtctccaccgacaaggtcgacaccgaaatcccatccccagtagcaggcaccatcgtggagatccttgcagacgaagacgacaccgtcgacgtcggcgcagtcatcgcccgcatcggtgacgcaaacgcagctgcagcacctggcgaagagaaagcagcacctgccgaagaggaagagccaaagcaggaagagccaaagaaggaagagccaaagaaggaagcagctactacacctgctgcggcatccgcaactgtgtccgcttctggcgacaacgttccatacgtcaccccactggtgcgcaagcttgctgaaaagcacggcgttgacttgaacaccgtgaccggtaccggtatcggtggccgtatccgcaagcaggatgttttggctgctgcgaacggcgaggctgcacctgctgaggctgctgctcctgtttccgcttggtccactaagtctgttgatcctgagaaggctaagctccgtggtaccactcagaaggtcaaccgcatccgtgagatcaccgcgatgaagaccgtcgaggctctgcagatttctgctcagctcacccagctgcacgaggtcgatatgactcgcgttgctgagctgcgtaagaagaacaagcccgcgttcatcgagaagcacggtgtgaacctcacttacctgccattcttcgtgaaggcagttgtcgaggctttggtttcccatccaaacgtcaacgcgtcttacaacgcgaagaccaaggagatgacctaccactcctccgttaacctctccatcgctgttgataccccagctggtctgttgaccccagtcattcacgatgctcaggatctctccatcccagagatcgcaaaggcaattgttgacctggctgatcgttcacgcaacaacaagctgaagccaaacgatctgtccggtggcaccttcaccatcaccaacattggttctgaaggcgcactgtctgataccccaatcctggttccaccacaggctggcatcttgggcaccggcgcgatcgtgaagcgtccagttgtcatcaccgaggatggaattgattccatcgcgatccgtcagatggtcttcctgccactgacctacgaccaccaggttgtagatggcgcagatgctggtcgcttcctgaccaccatcaaggaccgccttgagaccgctaacttcgaaggcgatctgcagctctaa

SEQ ID NO: 5 - DNA, 40 bp, Artificial Sequence
  aceF_1F
tgaattcgagctcggtacccacgacagacatctcattgac

SEQ ID NO: 6 - DNA, 33 bp, Artificial Sequence
  aceF_2R
agtctcatcagcatcgtcgattattgcaatgac

SEQ ID NO: 7 - DNA, 33 bp, Artificial Sequence
  aceF_3F
gtcattgcaataatcgacgatgctgatgagact

SEQ ID NO: 8 - DNA, 40 bp, Artificial Sequence
  aceF_4R
gtcgactctagaggatccccggtggagacctcaagaagtg

SEQ ID NO: 9 - DNA, 20 bp, Artificial Sequence
  aceF_5F
acgacagacatctcattgac

SEQ ID NO: 10 - DNA, 20 bp, Artificial Sequence
  aceF_6R
ggtggagacctcaagaagtg